European Patent Specification EP 3 539 982 B1, published February 19, 2025. Title: Engineered Antibody Constant Regions for Site-specific Conjugation and Methods and Uses Therefor. Applicant: Pfizer Inc Marquette, Kimberly Tchistiakova, Lioudmila Bennett, Eric Tumey, Lawrence Nathan Graziani, Edmund Bikker, Jack Calabro, Valerie. Application To be assigned. The sequence listing filed with the application follows.

SEQUENCE LISTING (205 sequences)

SEQ ID NO: 1 - protein, 330 aa, Homo sapiens
ASTKGPSVFPLAPSSKSTSGGTAALGCLVKDYFPEPVTVSWNSGALTSGVHTFPAVLQSSGLYSLSSVVTVPSSSLGTQTYICNVNHKPSNTKVDKKVEPKSCDKTHTCPPCPAPELLGGPSVFLFPPKPKDTLMISRTPEVTCVVVDVSHEDPEVKFNWYVDGVEVHNAKTKPREEQYNSTYRVVSVLTVLHQDWLNGKEYKCKVSNKALPAPIEKTISKAKGQPREPQVYTLPPSREEMTKNQVSLTCLVKGFYPSDIAVEWESNGQPENNYKTTPPVLDSDGSFFLYSKLTVDKSRWQQGNVFSCSVMHEALHNHYTQKSLSLSPGK

SEQ ID NO: 2 - DNA, 990 bp, Homo sapiens
gcgtcgaccaagggcccatcggtcttccccctggcaccctcctccaagagcacctctgggggcacagcggccctgggctgcctggtcaaggactacttccccgaaccggtgacggtgtcgtggaactcaggcgccctgaccagcggcgtgcacaccttcccggctgtcctacagtcctcaggactctactccctcagcagcgtggtgaccgtgccctccagcagcttgggcacccagacctacatctgcaacgtgaatcacaagcccagcaacaccaaggtggacaagaaagttgagcccaaatcttgtgacaaaactcacacatgcccaccgtgcccagcacctgaactcctggggggaccgtcagtcttcctcttccccccaaaacccaaggacaccctcatgatctcccggacccctgaggtcacatgcgtggtggtggacgtgagccacgaagaccctgaggtcaagttcaactggtacgtggacggcgtggaggtgcataatgccaagacaaagccgcgggaggagcagtacaacagcacgtaccgtgtggtcagcgtcctcaccgtcctgcaccaggactggctgaatggcaaggagtacaagtgcaaggtctccaacaaagccctcccagcccccatcgagaaaaccatctccaaagccaaagggcagccccgagaaccacaggtgtacaccctgcccccatcccgggaggagatgaccaagaaccaggtcagcctgacctgcctggtcaaaggcttctatcccagcgacatcgccgtggagtgggagagcaatgggcagccggagaacaactacaagaccacgcctcccgtgctggactccgacggctccttcttcctctatagcaagctcaccgtggacaagagcaggtggcagcaggggaacgtcttctcatgctccgtgatgcatgaggctctgcacaaccactacacgcagaagagcctctccctgtccccgggtaaa

SEQ ID NO: 3 - protein, 326 aa, HOMO SAPIENS
ASTKGPSVFPLAPCSRSTSESTAALGCLVKDYFPEPVTVSWNSGALTSGVHTFPAVLQSSGLYSLSSVVTVPSSNFGTQTYTCNVDHKPSNTKVDKTVERKCCVECPPCPAPPVAGPSVFLFPPKPKDTLMISRTPEVTCVVVDVSHEDPEVQFNWYVDGVEVHNAKTKPREEQFNSTFRVVSVLTVVHQDWLNGKEYKCKVSNKGLPAPIEKTISKTKGQPREPQVYTLPPSREEMTKNQVSLTCLVKGFYPSDISVEWESNGQPENNYKTTPPMLDSDGSFFLYSKLTVDKSRWQQGNVFSCSVMHEALHNHYTQKSLSLSPGK

SEQ ID NO: 4 - protein, 377 aa, HOMO SAPIENS
ASTKGPSVFPLAPCSRSTSGGTAALGCLVKDYFPEPVTVSWNSGALTSGVHTFPAVLQSSGLYSLSSVVTVPSSSLGTQTYTCNVNHKPSNTKVDKRVELKTPLGDTTHTCPRCPEPKSCDTPPPCPRCPEPKSCDTPPPCPRCPEPKSCDTPPPCPRCPAPELLGGPSVFLFPPKPKDTLMISRTPEVTCVVVDVSHEDPEVQFKWYVDGVEVHNAKTKPREEQYNSTFRVVSVLTVLHQDWLNGKEYKCKVSNKALPAPIEKTISKTKGQPREPQVYTLPPSREEMTKNQVSLTCLVKGFYPSDIAVEWESSGQPENNYNTTPPMLDSDGSFFLYSKLTVDKSRWQQGNIFSCSVMHEALHNRFTQKSLSLSPGK

SEQ ID NO: 5 - protein, 327 aa, HOMO SAPIENS
ASTKGPSVFPLAPCSRSTSESTAALGCLVKDYFPEPVTVSWNSGALTSGVHTFPAVLQSSGLYSLSSVVTVPSSSLGTKTYTCNVDHKPSNTKVDKRVESKYGPPCPSCPAPEFLGGPSVFLFPPKPKDTLMISRTPEVTCVVVDVSQEDPEVQFNWYVDGVEVHNAKTKPREEQFNSTYRVVSVLTVLHQDWLNGKEYKCKVSNKGLPSSIEKTISKAKGQPREPQVYTLPPSQEEMTKNQVSLTCLVKGFYPSDIAVEWESNGQPENNYKTTPPVLDSDGSFFLYSRLTVDKSRWQEGNVFSCSVMHEALHNHYTQKSLSLSLGK

SEQ ID NO: 6 - protein, 330 aa, Artificial Sequence
  IgG1-K246C
ASTKGPSVFPLAPSSKSTSGGTAALGCLVKDYFPEPVTVSWNSGALTSGVHTFPAVLQSSGLYSLSSVVTVPSSSLGTQTYICNVNHKPSNTKVDKKVEPKSCDKTHTCPPCPAPELLGGPSVFLFPPCPKDTLMISRTPEVTCVVVDVSHEDPEVKFNWYVDGVEVHNAKTKPREEQYNSTYRVVSVLTVLHQDWLNGKEYKCKVSNKALPAPIEKTISKAKGQPREPQVYTLPPSREEMTKNQVSLTCLVKGFYPSDIAVEWESNGQPENNYKTTPPVLDSDGSFFLYSKLTVDKSRWQQGNVFSCSVMHEALHNHYTQKSLSLSPGK

SEQ ID NO: 7 - protein, 330 aa, Artificial Sequence
  IgG1-D249C
ASTKGPSVFPLAPSSKSTSGGTAALGCLVKDYFPEPVTVSWNSGALTSGVHTFPAVLQSSGLYSLSSVVTVPSSSLGTQTYICNVNHKPSNTKVDKKVEPKSCDKTHTCPPCPAPELLGGPSVFLFPPKPKCTLMISRTPEVTCVVVDVSHEDPEVKFNWYVDGVEVHNAKTKPREEQYNSTYRVVSVLTVLHQDWLNGKEYKCKVSNKALPAPIEKTISKAKGQPREPQVYTLPPSREEMTKNQVSLTCLVKGFYPSDIAVEWESNGQPENNYKTTPPVLDSDGSFFLYSKLTVDKSRWQQGNVFSCSVMHEALHNHYTQKSLSLSPGK

SEQ ID NO: 8 - protein, 330 aa, Artificial Sequence
  human IgG1-S254C
ASTKGPSVFPLAPSSKSTSGGTAALGCLVKDYFPEPVTVSWNSGALTSGVHTFPAVLQSSGLYSLSSVVTVPSSSLGTQTYICNVNHKPSNTKVDKKVEPKSCDKTHTCPPCPAPELLGGPSVFLFPPKPKDTLMICRTPEVTCVVVDVSHEDPEVKFNWYVDGVEVHNAKTKPREEQYNSTYRVVSVLTVLHQDWLNGKEYKCKVSNKALPAPIEKTISKAKGQPREPQVYTLPPSREEMTKNQVSLTCLVKGFYPSDIAVEWESNGQPENNYKTTPPVLDSDGSFFLYSKLTVDKSRWQQGNVFSCSVMHEALHNHYTQKSLSLSPGK

SEQ ID NO: 9 - protein, 330 aa, Artificial Sequence
  human IgG1-D265C
ASTKGPSVFPLAPSSKSTSGGTAALGCLVKDYFPEPVTVSWNSGALTSGVHTFPAVLQSSGLYSLSSVVTVPSSSLGTQTYICNVNHKPSNTKVDKKVEPKSCDKTHTCPPCPAPELLGGPSVFLFPPKPKDTLMISRTPEVTCVVVCVSHEDPEVKFNWYVDGVEVHNAKTKPREEQYNSTYRVVSVLTVLHQDWLNGKEYKCKVSNKALPAPIEKTISKAKGQPREPQVYTLPPSREEMTKNQVSLTCLVKGFYPSDIAVEWESNGQPENNYKTTPPVLDSDGSFFLYSKLTVDKSRWQQGNVFSCSVMHEALHNHYTQKSLSLSPGK

SEQ ID NO: 10 - protein, 330 aa, Artificial Sequence
  human IgG1-S267C
ASTKGPSVFPLAPSSKSTSGGTAALGCLVKDYFPEPVTVSWNSGALTSGVHTFPAVLQSSGLYSLSSVVTVPSSSLGTQTYICNVNHKPSNTKVDKKVEPKSCDKTHTCPPCPAPELLGGPSVFLFPPKPKDTLMISRTPEVTCVVVDVCHEDPEVKFNWYVDGVEVHNAKTKPREEQYNSTYRVVSVLTVLHQDWLNGKEYKCKVSNKALPAPIEKTISKAKGQPREPQVYTLPPSREEMTKNQVSLTCLVKGFYPSDIAVEWESNGQPENNYKTTPPVLDSDGSFFLYSKLTVDKSRWQQGNVFSCSVMHEALHNHYTQKSLSLSPGK

SEQ ID NO: 11 - protein, 330 aa, Artificial Sequence
  human IgG1-D270C
ASTKGPSVFPLAPSSKSTSGGTAALGCLVKDYFPEPVTVSWNSGALTSGVHTFPAVLQSSGLYSLSSVVTVPSSSLGTQTYICNVNHKPSNTKVDKKVEPKSCDKTHTCPPCPAPELLGGPSVFLFPPKPKDTLMISRTPEVTCVVVDVSHECPEVKFNWYVDGVEVHNAKTKPREEQYNSTYRVVSVLTVLHQDWLNGKEYKCKVSNKALPAPIEKTISKAKGQPREPQVYTLPPSREEMTKNQVSLTCLVKGFYPSDIAVEWESNGQPENNYKTTPPVLDSDGSFFLYSKLTVDKSRWQQGNVFSCSVMHEALHNHYTQKSLSLSPGK

SEQ ID NO: 12 - protein, 330 aa, human IgG1-N276C
ASTKGPSVFPLAPSSKSTSGGTAALGCLVKDYFPEPVTVSWNSGALTSGVHTFPAVLQSSGLYSLSSVVTVPSSSLGTQTYICNVNHKPSNTKVDKKVEPKSCDKTHTCPPCPAPELLGGPSVFLFPPKPKDTLMISRTPEVTCVVVDVSHEDPEVKFCWYVDGVEVHNAKTKPREEQYNSTYRVVSVLTVLHQDWLNGKEYKCKVSNKALPAPIEKTISKAKGQPREPQVYTLPPSREEMTKNQVSLTCLVKGFYPSDIAVEWESNGQPENNYKTTPPVLDSDGSFFLYSKLTVDKSRWQQGNVFSCSVMHEALHNHYTQKSLSLSPGK

SEQ ID NO: 13 - protein, 330 aa, Artificial Sequence
  human IgG1-Y278C
ASTKGPSVFPLAPSSKSTSGGTAALGCLVKDYFPEPVTVSWNSGALTSGVHTFPAVLQSSGLYSLSSVVTVPSSSLGTQTYICNVNHKPSNTKVDKKVEPKSCDKTHTCPPCPAPELLGGPSVFLFPPKPKDTLMISRTPEVTCVVVDVSHEDPEVKFNWCVDGVEVHNAKTKPREEQYNSTYRVVSVLTVLHQDWLNGKEYKCKVSNKALPAPIEKTISKAKGQPREPQVYTLPPSREEMTKNQVSLTCLVKGFYPSDIAVEWESNGQPENNYKTTPPVLDSDGSFFLYSKLTVDKSRWQQGNVFSCSVMHEALHNHYTQKSLSLSPGK

SEQ ID NO: 14 - protein, 330 aa, Artificial Sequence
  human IgG1-E283C
ASTKGPSVFPLAPSSKSTSGGTAALGCLVKDYFPEPVTVSWNSGALTSGVHTFPAVLQSSGLYSLSSVVTVPSSSLGTQTYICNVNHKPSNTKVDKKVEPKSCDKTHTCPPCPAPELLGGPSVFLFPPKPKDTLMISRTPEVTCVVVDVSHEDPEVKFNWYVDGVCVHNAKTKPREEQYNSTYRVVSVLTVLHQDWLNGKEYKCKVSNKALPAPIEKTISKAKGQPREPQVYTLPPSREEMTKNQVSLTCLVKGFYPSDIAVEWESNGQPENNYKTTPPVLDSDGSFFLYSKLTVDKSRWQQGNVFSCSVMHEALHNHYTQKSLSLSPGK

SEQ ID NO: 15 - protein, 330 aa, Artificial Sequence
  IgG1-V284C
ASTKGPSVFPLAPSSKSTSGGTAALGCLVKDYFPEPVTVSWNSGALTSGVHTFPAVLQSSGLYSLSSVVTVPSSSLGTQTYICNVNHKPSNTKVDKKVEPKSCDKTHTCPPCPAPELLGGPSVFLFPPKPKDTLMISRTPEVTCVVVDVSHEDPEVKFNWYVDGVECHNAKTKPREEQYNSTYRVVSVLTVLHQDWLNGKEYKCKVSNKALPAPIEKTISKAKGQPREPQVYTLPPSREEMTKNQVSLTCLVKGFYPSDIAVEWESNGQPENNYKTTPPVLDSDGSFFLYSKLTVDKSRWQQGNVFSCSVMHEALHNHYTQKSLSLSPGK

SEQ ID NO: 16 - protein, 330 aa, Artificial Sequence
  human IgG1-A287C
ASTKGPSVFPLAPSSKSTSGGTAALGCLVKDYFPEPVTVSWNSGALTSGVHTFPAVLQSSGLYSLSSVVTVPSSSLGTQTYICNVNHKPSNTKVDKKVEPKSCDKTHTCPPCPAPELLGGPSVFLFPPKPKDTLMISRTPEVTCVVVDVSHEDPEVKFNWYVDGVEVHNCKTKPREEQYNSTYRVVSVLTVLHQDWLNGKEYKCKVSNKALPAPIEKTISKAKGQPREPQVYTLPPSREEMTKNQVSLTCLVKGFYPSDIAVEWESNGQPENNYKTTPPVLDSDGSFFLYSKLTVDKSRWQQGNVFSCSVMHEALHNHYTQKSLSLSPGK

SEQ ID NO: 17 - protein, 330 aa, Artificial Sequence
  human IgG1-R292C
ASTKGPSVFPLAPSSKSTSGGTAALGCLVKDYFPEPVTVSWNSGALTSGVHTFPAVLQSSGLYSLSSVVTVPSSSLGTQTYICNVNHKPSNTKVDKKVEPKSCDKTHTCPPCPAPELLGGPSVFLFPPKPKDTLMISRTPEVTCVVVDVSHEDPEVKFNWYVDGVEVHNAKTKPCEEQYNSTYRVVSVLTVLHQDWLNGKEYKCKVSNKALPAPIEKTISKAKGQPREPQVYTLPPSREEMTKNQVSLTCLVKGFYPSDIAVEWESNGQPENNYKTTPPVLDSDGSFFLYSKLTVDKSRWQQGNVFSCSVMHEALHNHYTQKSLSLSPGK

SEQ ID NO: 18 - protein, 330 aa, Artificial Sequence
  human IgG1-E293C
ASTKGPSVFPLAPSSKSTSGGTAALGCLVKDYFPEPVTVSWNSGALTSGVHTFPAVLQSSGLYSLSSVVTVPSSSLGTQTYICNVNHKPSNTKVDKKVEPKSCDKTHTCPPCPAPELLGGPSVFLFPPKPKDTLMISRTPEVTCVVVDVSHEDPEVKFNWYVDGVEVHNAKTKPRCEQYNSTYRVVSVLTVLHQDWLNGKEYKCKVSNKALPAPIEKTISKAKGQPREPQVYTLPPSREEMTKNQVSLTCLVKGFYPSDIAVEWESNGQPENNYKTTPPVLDSDGSFFLYSKLTVDKSRWQQGNVFSCSVMHEALHNHYTQKSLSLSPGK

SEQ ID NO: 19 - protein, 330 aa, Artificial Sequence
  human IgG1-E294C
ASTKGPSVFPLAPSSKSTSGGTAALGCLVKDYFPEPVTVSWNSGALTSGVHTFPAVLQSSGLYSLSSVVTVPSSSLGTQTYICNVNHKPSNTKVDKKVEPKSCDKTHTCPPCPAPELLGGPSVFLFPPKPKDTLMISRTPEVTCVVVDVSHEDPEVKFNWYVDGVEVHNAKTKPRECQYNSTYRVVSVLTVLHQDWLNGKEYKCKVSNKALPAPIEKTISKAKGQPREPQVYTLPPSREEMTKNQVSLTCLVKGFYPSDIAVEWESNGQPENNYKTTPPVLDSDGSFFLYSKLTVDKSRWQQGNVFSCSVMHEALHNHYTQKSLSLSPGK

SEQ ID NO: 20 - protein, 330 aa, Artificial Sequence
  human IgG1-Y300C
ASTKGPSVFPLAPSSKSTSGGTAALGCLVKDYFPEPVTVSWNSGALTSGVHTFPAVLQSSGLYSLSSVVTVPSSSLGTQTYICNVNHKPSNTKVDKKVEPKSCDKTHTCPPCPAPELLGGPSVFLFPPKPKDTLMISRTPEVTCVVVDVSHEDPEVKFNWYVDGVEVHNAKTKPREEQYNSTCRVVSVLTVLHQDWLNGKEYKCKVSNKALPAPIEKTISKAKGQPREPQVYTLPPSREEMTKNQVSLTCLVKGFYPSDIAVEWESNGQPENNYKTTPPVLDSDGSFFLYSKLTVDKSRWQQGNVFSCSVMHEALHNHYTQKSLSLSPGK

SEQ ID NO: 21 - protein, 330 aa, Artificial Sequence
  human IgG1-V302C
ASTKGPSVFPLAPSSKSTSGGTAALGCLVKDYFPEPVTVSWNSGALTSGVHTFPAVLQSSGLYSLSSVVTVPSSSLGTQTYICNVNHKPSNTKVDKKVEPKSCDKTHTCPPCPAPELLGGPSVFLFPPKPKDTLMISRTPEVTCVVVDVSHEDPEVKFNWYVDGVEVHNAKTKPREEQYNSTYRCVSVLTVLHQDWLNGKEYKCKVSNKALPAPIEKTISKAKGQPREPQVYTLPPSREEMTKNQVSLTCLVKGFYPSDIAVEWESNGQPENNYKTTPPVLDSDGSFFLYSKLTVDKSRWQQGNVFSCSVMHEALHNHYTQKSLSLSPGK

SEQ ID NO: 22 - protein, 330 aa, Artificial Sequence
  human IgG1-V303C
ASTKGPSVFPLAPSSKSTSGGTAALGCLVKDYFPEPVTVSWNSGALTSGVHTFPAVLQSSGLYSLSSVVTVPSSSLGTQTYICNVNHKPSNTKVDKKVEPKSCDKTHTCPPCPAPELLGGPSVFLFPPKPKDTLMISRTPEVTCVVVDVSHEDPEVKFNWYVDGVEVHNAKTKPREEQYNSTYRVCSVLTVLHQDWLNGKEYKCKVSNKALPAPIEKTISKAKGQPREPQVYTLPPSREEMTKNQVSLTCLVKGFYPSDIAVEWESNGQPENNYKTTPPVLDSDGSFFLYSKLTVDKSRWQQGNVFSCSVMHEALHNHYTQKSLSLSPGK

SEQ ID NO: 23 - protein, 330 aa, Artificial Sequence
  human IgG1-L314C
ASTKGPSVFPLAPSSKSTSGGTAALGCLVKDYFPEPVTVSWNSGALTSGVHTFPAVLQSSGLYSLSSVVTVPSSSLGTQTYICNVNHKPSNTKVDKKVEPKSCDKTHTCPPCPAPELLGGPSVFLFPPKPKDTLMISRTPEVTCVVVDVSHEDPEVKFNWYVDGVEVHNAKTKPREEQYNSTYRVVSVLTVLHQDWCNGKEYKCKVSNKALPAPIEKTISKAKGQPREPQVYTLPPSREEMTKNQVSLTCLVKGFYPSDIAVEWESNGQPENNYKTTPPVLDSDGSFFLYSKLTVDKSRWQQGNVFSCSVMHEALHNHYTQKSLSLSPGK

SEQ ID NO: 24 - protein, 330 aa, Artificial Sequence
  human IgG1-N315C
ASTKGPSVFPLAPSSKSTSGGTAALGCLVKDYFPEPVTVSWNSGALTSGVHTFPAVLQSSGLYSLSSVVTVPSSSLGTQTYICNVNHKPSNTKVDKKVEPKSCDKTHTCPPCPAPELLGGPSVFLFPPKPKDTLMISRTPEVTCVVVDVSHEDPEVKFNWYVDGVEVHNAKTKPREEQYNSTYRVVSVLTVLHQDWLCGKEYKCKVSNKALPAPIEKTISKAKGQPREPQVYTLPPSREEMTKNQVSLTCLVKGFYPSDIAVEWESNGQPENNYKTTPPVLDSDGSFFLYSKLTVDKSRWQQGNVFSCSVMHEALHNHYTQKSLSLSPGK

SEQ ID NO: 25 - protein, 330 aa, Artificial Sequence
  human IgG1-E318C
ASTKGPSVFPLAPSSKSTSGGTAALGCLVKDYFPEPVTVSWNSGALTSGVHTFPAVLQSSGLYSLSSVVTVPSSSLGTQTYICNVNHKPSNTKVDKKVEPKSCDKTHTCPPCPAPELLGGPSVFLFPPKPKDTLMISRTPEVTCVVVDVSHEDPEVKFNWYVDGVEVHNAKTKPREEQYNSTYRVVSVLTVLHQDWLNGKCYKCKVSNKALPAPIEKTISKAKGQPREPQVYTLPPSREEMTKNQVSLTCLVKGFYPSDIAVEWESNGQPENNYKTTPPVLDSDGSFFLYSKLTVDKSRWQQGNVFSCSVMHEALHNHYTQKSLSLSPGK

SEQ ID NO: 26 - protein, 330 aa, Artificial Sequence
  human IgG1-K320C
ASTKGPSVFPLAPSSKSTSGGTAALGCLVKDYFPEPVTVSWNSGALTSGVHTFPAVLQSSGLYSLSSVVTVPSSSLGTQTYICNVNHKPSNTKVDKKVEPKSCDKTHTCPPCPAPELLGGPSVFLFPPKPKDTLMISRTPEVTCVVVDVSHEDPEVKFNWYVDGVEVHNAKTKPREEQYNSTYRVVSVLTVLHQDWLNGKEYCCKVSNKALPAPIEKTISKAKGQPREPQVYTLPPSREEMTKNQVSLTCLVKGFYPSDIAVEWESNGQPENNYKTTPPVLDSDGSFFLYSKLTVDKSRWQQGNVFSCSVMHEALHNHYTQKSLSLSPGK

SEQ ID NO: 27 - protein, 330 aa, Artificial Sequence
  human IgG1-A327C
ASTKGPSVFPLAPSSKSTSGGTAALGCLVKDYFPEPVTVSWNSGALTSGVHTFPAVLQSSGLYSLSSVVTVPSSSLGTQTYICNVNHKPSNTKVDKKVEPKSCDKTHTCPPCPAPELLGGPSVFLFPPKPKDTLMISRTPEVTCVVVDVSHEDPEVKFNWYVDGVEVHNAKTKPREEQYNSTYRVVSVLTVLHQDWLNGKEYKCKVSNKCLPAPIEKTISKAKGQPREPQVYTLPPSREEMTKNQVSLTCLVKGFYPSDIAVEWESNGQPENNYKTTPPVLDSDGSFFLYSKLTVDKSRWQQGNVFSCSVMHEALHNHYTQKSLSLSPGK

SEQ ID NO: 28 - protein, 330 aa, Artificial Sequence
  human IgG1-I332C
ASTKGPSVFPLAPSSKSTSGGTAALGCLVKDYFPEPVTVSWNSGALTSGVHTFPAVLQSSGLYSLSSVVTVPSSSLGTQTYICNVNHKPSNTKVDKKVEPKSCDKTHTCPPCPAPELLGGPSVFLFPPKPKDTLMISRTPEVTCVVVDVSHEDPEVKFNWYVDGVEVHNAKTKPREEQYNSTYRVVSVLTVLHQDWLNGKEYKCKVSNKALPAPCEKTISKAKGQPREPQVYTLPPSREEMTKNQVSLTCLVKGFYPSDIAVEWESNGQPENNYKTTPPVLDSDGSFFLYSKLTVDKSRWQQGNVFSCSVMHEALHNHYTQKSLSLSPGK

SEQ ID NO: 29 - protein, 330 aa, Artificial Sequence
  human IgG1-E333C
ASTKGPSVFPLAPSSKSTSGGTAALGCLVKDYFPEPVTVSWNSGALTSGVHTFPAVLQSSGLYSLSSVVTVPSSSLGTQTYICNVNHKPSNTKVDKKVEPKSCDKTHTCPPCPAPELLGGPSVFLFPPKPKDTLMISRTPEVTCVVVDVSHEDPEVKFNWYVDGVEVHNAKTKPREEQYNSTYRVVSVLTVLHQDWLNGKEYKCKVSNKALPAPICKTISKAKGQPREPQVYTLPPSREEMTKNQVSLTCLVKGFYPSDIAVEWESNGQPENNYKTTPPVLDSDGSFFLYSKLTVDKSRWQQGNVFSCSVMHEALHNHYTQKSLSLSPGK

SEQ ID NO: 30 - protein, 330 aa, Artificial Sequence
  human IgG1-K334C
ASTKGPSVFPLAPSSKSTSGGTAALGCLVKDYFPEPVTVSWNSGALTSGVHTFPAVLQSSGLYSLSSVVTVPSSSLGTQTYICNVNHKPSNTKVDKKVEPKSCDKTHTCPPCPAPELLGGPSVFLFPPKPKDTLMISRTPEVTCVVVDVSHEDPEVKFNWYVDGVEVHNAKTKPREEQYNSTYRVVSVLTVLHQDWLNGKEYKCKVSNKALPAPIECTISKAKGQPREPQVYTLPPSREEMTKNQVSLTCLVKGFYPSDIAVEWESNGQPENNYKTTPPVLDSDGSFFLYSKLTVDKSRWQQGNVFSCSVMHEALHNHYTQKSLSLSPGK

SEQ ID NO: 31 - protein, 330 aa, Artificial Sequence
  human IgG1-I336C
ASTKGPSVFPLAPSSKSTSGGTAALGCLVKDYFPEPVTVSWNSGALTSGVHTFPAVLQSSGLYSLSSVVTVPSSSLGTQTYICNVNHKPSNTKVDKKVEPKSCDKTHTCPPCPAPELLGGPSVFLFPPKPKDTLMISRTPEVTCVVVDVSHEDPEVKFNWYVDGVEVHNAKTKPREEQYNSTYRVVSVLTVLHQDWLNGKEYKCKVSNKALPAPIEKTCSKAKGQPREPQVYTLPPSREEMTKNQVSLTCLVKGFYPSDIAVEWESNGQPENNYKTTPPVLDSDGSFFLYSKLTVDKSRWQQGNVFSCSVMHEALHNHYTQKSLSLSPGK

SEQ ID NO: 32 - protein, 330 aa, Artificial Sequence
  human IgG1-E345C
ASTKGPSVFPLAPSSKSTSGGTAALGCLVKDYFPEPVTVSWNSGALTSGVHTFPAVLQSSGLYSLSSVVTVPSSSLGTQTYICNVNHKPSNTKVDKKVEPKSCDKTHTCPPCPAPELLGGPSVFLFPPKPKDTLMISRTPEVTCVVVDVSHEDPEVKFNWYVDGVEVHNAKTKPREEQYNSTYRVVSVLTVLHQDWLNGKEYKCKVSNKALPAPIEKTISKAKGQPRCPQVYTLPPSREEMTKNQVSLTCLVKGFYPSDIAVEWESNGQPENNYKTTPPVLDSDGSFFLYSKLTVDKSRWQQGNVFSCSVMHEALHNHYTQKSLSLSPGK

SEQ ID NO: 33 - protein, 330 aa, Artificial Sequence
  33 human GG IgG1-Q347C
ASTKGPSVFPLAPSSKSTSGGTAALGCLVKDYFPEPVTVSWNSGALTSGVHTFPAVLQSSGLYSLSSVVTVPSSSLGTQTYICNVNHKPSNTKVDKKVEPKSCDKTHTCPPCPAPELLGGPSVFLFPPKPKDTLMISRTPEVTCVVVDVSHEDPEVKFNWYVDGVEVHNAKTKPREEQYNSTYRVVSVLTVLHQDWLNGKEYKCKVSNKALPAPIEKTISKAKGQPREPCVYTLPPSREEMTKNQVSLTCLVKGFYPSDIAVEWESNGQPENNYKTTPPVLDSDGSFFLYSKLTVDKSRWQQGNVFSCSVMHEALHNHYTQKSLSLSPGK

SEQ ID NO: 34 - protein, 330 aa, Artificial Sequence
  34 human HH  IgG1-S354C
ASTKGPSVFPLAPSSKSTSGGTAALGCLVKDYFPEPVTVSWNSGALTSGVHTFPAVLQSSGLYSLSSVVTVPSSSLGTQTYICNVNHKPSNTKVDKKVEPKSCDKTHTCPPCPAPELLGGPSVFLFPPKPKDTLMISRTPEVTCVVVDVSHEDPEVKFNWYVDGVEVHNAKTKPREEQYNSTYRVVSVLTVLHQDWLNGKEYKCKVSNKALPAPIEKTISKAKGQPREPQVYTLPPCREEMTKNQVSLTCLVKGFYPSDIAVEWESNGQPENNYKTTPPVLDSDGSFFLYSKLTVDKSRWQQGNVFSCSVMHEALHNHYTQKSLSLSPGK

SEQ ID NO: 35 - protein, 330 aa, Artificial Sequence
  35 human II IgG1-R355C
ASTKGPSVFPLAPSSKSTSGGTAALGCLVKDYFPEPVTVSWNSGALTSGVHTFPAVLQSSGLYSLSSVVTVPSSSLGTQTYICNVNHKPSNTKVDKKVEPKSCDKTHTCPPCPAPELLGGPSVFLFPPKPKDTLMISRTPEVTCVVVDVSHEDPEVKFNWYVDGVEVHNAKTKPREEQYNSTYRVVSVLTVLHQDWLNGKEYKCKVSNKALPAPIEKTISKAKGQPREPQVYTLPPSCEEMTKNQVSLTCLVKGFYPSDIAVEWESNGQPENNYKTTPPVLDSDGSFFLYSKLTVDKSRWQQGNVFSCSVMHEALHNHYTQKSLSLSPGK

SEQ ID NO: 36 - protein, 330 aa, Artificial Sequence
  36 human JJ  IgG1-M358C
ASTKGPSVFPLAPSSKSTSGGTAALGCLVKDYFPEPVTVSWNSGALTSGVHTFPAVLQSSGLYSLSSVVTVPSSSLGTQTYICNVNHKPSNTKVDKKVEPKSCDKTHTCPPCPAPELLGGPSVFLFPPKPKDTLMISRTPEVTCVVVDVSHEDPEVKFNWYVDGVEVHNAKTKPREEQYNSTYRVVSVLTVLHQDWLNGKEYKCKVSNKALPAPIEKTISKAKGQPREPQVYTLPPSREECTKNQVSLTCLVKGFYPSDIAVEWESNGQPENNYKTTPPVLDSDGSFFLYSKLTVDKSRWQQGNVFSCSVMHEALHNHYTQKSLSLSPGK

SEQ ID NO: 37 - protein, 330 aa, Artificial Sequence
  37 human KK. IgG1-T359C
ASTKGPSVFPLAPSSKSTSGGTAALGCLVKDYFPEPVTVSWNSGALTSGVHTFPAVLQSSGLYSLSSVVTVPSSSLGTQTYICNVNHKPSNTKVDKKVEPKSCDKTHTCPPCPAPELLGGPSVFLFPPKPKDTLMISRTPEVTCVVVDVSHEDPEVKFNWYVDGVEVHNAKTKPREEQYNSTYRVVSVLTVLHQDWLNGKEYKCKVSNKALPAPIEKTISKAKGQPREPQVYTLPPSREEMCKNQVSLTCLVKGFYPSDIAVEWESNGQPENNYKTTPPVLDSDGSFFLYSKLTVDKSRWQQGNVFSCSVMHEALHNHYTQKSLSLSPGK

SEQ ID NO: 38 - protein, 330 aa, Artificial Sequence
  38 human LL  IgG1-K360C
ASTKGPSVFPLAPSSKSTSGGTAALGCLVKDYFPEPVTVSWNSGALTSGVHTFPAVLQSSGLYSLSSVVTVPSSSLGTQTYICNVNHKPSNTKVDKKVEPKSCDKTHTCPPCPAPELLGGPSVFLFPPKPKDTLMISRTPEVTCVVVDVSHEDPEVKFNWYVDGVEVHNAKTKPREEQYNSTYRVVSVLTVLHQDWLNGKEYKCKVSNKALPAPIEKTISKAKGQPREPQVYTLPPSREEMTCNQVSLTCLVKGFYPSDIAVEWESNGQPENNYKTTPPVLDSDGSFFLYSKLTVDKSRWQQGNVFSCSVMHEALHNHYTQKSLSLSPGK

SEQ ID NO: 39 - protein, 330 aa, Artificial Sequence
  MM  IgG1-N361C
ASTKGPSVFPLAPSSKSTSGGTAALGCLVKDYFPEPVTVSWNSGALTSGVHTFPAVLQSSGLYSLSSVVTVPSSSLGTQTYICNVNHKPSNTKVDKKVEPKSCDKTHTCPPCPAPELLGGPSVFLFPPKPKDTLMISRTPEVTCVVVDVSHEDPEVKFNWYVDGVEVHNAKTKPREEQYNSTYRVVSVLTVLHQDWLNGKEYKCKVSNKALPAPIEKTISKAKGQPREPQVYTLPPSREEMTKCQVSLTCLVKGFYPSDIAVEWESNGQPENNYKTTPPVLDSDGSFFLYSKLTVDKSRWQQGNVFSCSVMHEALHNHYTQKSLSLSPGK

SEQ ID NO: 40 - protein, 330 aa, Artificial Sequence
  40 human NN  IgG1-Q362C
ASTKGPSVFPLAPSSKSTSGGTAALGCLVKDYFPEPVTVSWNSGALTSGVHTFPAVLQSSGLYSLSSVVTVPSSSLGTQTYICNVNHKPSNTKVDKKVEPKSCDKTHTCPPCPAPELLGGPSVFLFPPKPKDTLMISRTPEVTCVVVDVSHEDPEVKFNWYVDGVEVHNAKTKPREEQYNSTYRVVSVLTVLHQDWLNGKEYKCKVSNKALPAPIEKTISKAKGQPREPQVYTLPPSREEMTKNCVSLTCLVKGFYPSDIAVEWESNGQPENNYKTTPPVLDSDGSFFLYSKLTVDKSRWQQGNVFSCSVMHEALHNHYTQKSLSLSPGK

SEQ ID NO: 41 - protein, 330 aa, Artificial Sequence
  41 human OO.  IgG1-K370C
ASTKGPSVFPLAPSSKSTSGGTAALGCLVKDYFPEPVTVSWNSGALTSGVHTFPAVLQSSGLYSLSSVVTVPSSSLGTQTYICNVNHKPSNTKVDKKVEPKSCDKTHTCPPCPAPELLGGPSVFLFPPKPKDTLMISRTPEVTCVVVDVSHEDPEVKFNWYVDGVEVHNAKTKPREEQYNSTYRVVSVLTVLHQDWLNGKEYKCKVSNKALPAPIEKTISKAKGQPREPQVYTLPPSREEMTKNQVSLTCLVCGFYPSDIAVEWESNGQPENNYKTTPPVLDSDGSFFLYSKLTVDKSRWQQGNVFSCSVMHEALHNHYTQKSLSLSPGK

SEQ ID NO: 42 - protein, 330 aa, Artificial Sequence
  42 human PP.  IgG1-Y373C
ASTKGPSVFPLAPSSKSTSGGTAALGCLVKDYFPEPVTVSWNSGALTSGVHTFPAVLQSSGLYSLSSVVTVPSSSLGTQTYICNVNHKPSNTKVDKKVEPKSCDKTHTCPPCPAPELLGGPSVFLFPPKPKDTLMISRTPEVTCVVVDVSHEDPEVKFNWYVDGVEVHNAKTKPREEQYNSTYRVVSVLTVLHQDWLNGKEYKCKVSNKALPAPIEKTISKAKGQPREPQVYTLPPSREEMTKNQVSLTCLVKGFCPSDIAVEWESNGQPENNYKTTPPVLDSDGSFFLYSKLTVDKSRWQQGNVFSCSVMHEALHNHYTQKSLSLSPGK

SEQ ID NO: 43 - protein, 330 aa, Artificial Sequence
  43 human QQ.  IgG1-D376C
ASTKGPSVFPLAPSSKSTSGGTAALGCLVKDYFPEPVTVSWNSGALTSGVHTFPAVLQSSGLYSLSSVVTVPSSSLGTQTYICNVNHKPSNTKVDKKVEPKSCDKTHTCPPCPAPELLGGPSVFLFPPKPKDTLMISRTPEVTCVVVDVSHEDPEVKFNWYVDGVEVHNAKTKPREEQYNSTYRVVSVLTVLHQDWLNGKEYKCKVSNKALPAPIEKTISKAKGQPREPQVYTLPPSREEMTKNQVSLTCLVKGFYPSCIAVEWESNGQPENNYKTTPPVLDSDGSFFLYSKLTVDKSRWQQGNVFSCSVMHEALHNHYTQKSLSLSPGK

SEQ ID NO: 44 - protein, 330 aa, Artificial Sequence
  44 human RR.  IgG1-A378C
ASTKGPSVFPLAPSSKSTSGGTAALGCLVKDYFPEPVTVSWNSGALTSGVHTFPAVLQSSGLYSLSSVVTVPSSSLGTQTYICNVNHKPSNTKVDKKVEPKSCDKTHTCPPCPAPELLGGPSVFLFPPKPKDTLMISRTPEVTCVVVDVSHEDPEVKFNWYVDGVEVHNAKTKPREEQYNSTYRVVSVLTVLHQDWLNGKEYKCKVSNKALPAPIEKTISKAKGQPREPQVYTLPPSREEMTKNQVSLTCLVKGFYPSDICVEWESNGQPENNYKTTPPVLDSDGSFFLYSKLTVDKSRWQQGNVFSCSVMHEALHNHYTQKSLSLSPGK

SEQ ID NO: 45 - protein, 330 aa, Artificial Sequence
  45 human SS.  IgG1-E380C
ASTKGPSVFPLAPSSKSTSGGTAALGCLVKDYFPEPVTVSWNSGALTSGVHTFPAVLQSSGLYSLSSVVTVPSSSLGTQTYICNVNHKPSNTKVDKKVEPKSCDKTHTCPPCPAPELLGGPSVFLFPPKPKDTLMISRTPEVTCVVVDVSHEDPEVKFNWYVDGVEVHNAKTKPREEQYNSTYRVVSVLTVLHQDWLNGKEYKCKVSNKALPAPIEKTISKAKGQPREPQVYTLPPSREEMTKNQVSLTCLVKGFYPSDIAVCWESNGQPENNYKTTPPVLDSDGSFFLYSKLTVDKSRWQQGNVFSCSVMHEALHNHYTQKSLSLSPGK

SEQ ID NO: 46 - protein, 330 aa, Artificial Sequence
  46 human TT.  IgG1-E382C
ASTKGPSVFPLAPSSKSTSGGTAALGCLVKDYFPEPVTVSWNSGALTSGVHTFPAVLQSSGLYSLSSVVTVPSSSLGTQTYICNVNHKPSNTKVDKKVEPKSCDKTHTCPPCPAPELLGGPSVFLFPPKPKDTLMISRTPEVTCVVVDVSHEDPEVKFNWYVDGVEVHNAKTKPREEQYNSTYRVVSVLTVLHQDWLNGKEYKCKVSNKALPAPIEKTISKAKGQPREPQVYTLPPSREEMTKNQVSLTCLVKGFYPSDIAVEWCSNGQPENNYKTTPPVLDSDGSFFLYSKLTVDKSRWQQGNVFSCSVMHEALHNHYTQKSLSLSPGK

SEQ ID NO: 47 - protein, 330 aa, Artificial Sequence
  47 human UU  IgG1-S383C
ASTKGPSVFPLAPSSKSTSGGTAALGCLVKDYFPEPVTVSWNSGALTSGVHTFPAVLQSSGLYSLSSVVTVPSSSLGTQTYICNVNHKPSNTKVDKKVEPKSCDKTHTCPPCPAPELLGGPSVFLFPPKPKDTLMISRTPEVTCVVVDVSHEDPEVKFNWYVDGVEVHNAKTKPREEQYNSTYRVVSVLTVLHQDWLNGKEYKCKVSNKALPAPIEKTISKAKGQPREPQVYTLPPSREEMTKNQVSLTCLVKGFYPSDIAVEWECNGQPENNYKTTPPVLDSDGSFFLYSKLTVDKSRWQQGNVFSCSVMHEALHNHYTQKSLSLSPGK

SEQ ID NO: 48 - protein, 330 aa, Artificial Sequence
  48 human VV  IgG1-N384C
ASTKGPSVFPLAPSSKSTSGGTAALGCLVKDYFPEPVTVSWNSGALTSGVHTFPAVLQSSGLYSLSSVVTVPSSSLGTQTYICNVNHKPSNTKVDKKVEPKSCDKTHTCPPCPAPELLGGPSVFLFPPKPKDTLMISRTPEVTCVVVDVSHEDPEVKFNWYVDGVEVHNAKTKPREEQYNSTYRVVSVLTVLHQDWLNGKEYKCKVSNKALPAPIEKTISKAKGQPREPQVYTLPPSREEMTKNQVSLTCLVKGFYPSDIAVEWESCGQPENNYKTTPPVLDSDGSFFLYSKLTVDKSRWQQGNVFSCSVMHEALHNHYTQKSLSLSPGK

SEQ ID NO: 49 - protein, 330 aa, Artificial Sequence
  49 human WW.  IgG1-Q386C
ASTKGPSVFPLAPSSKSTSGGTAALGCLVKDYFPEPVTVSWNSGALTSGVHTFPAVLQSSGLYSLSSVVTVPSSSLGTQTYICNVNHKPSNTKVDKKVEPKSCDKTHTCPPCPAPELLGGPSVFLFPPKPKDTLMISRTPEVTCVVVDVSHEDPEVKFNWYVDGVEVHNAKTKPREEQYNSTYRVVSVLTVLHQDWLNGKEYKCKVSNKALPAPIEKTISKAKGQPREPQVYTLPPSREEMTKNQVSLTCLVKGFYPSDIAVEWESNGCPENNYKTTPPVLDSDGSFFLYSKLTVDKSRWQQGNVFSCSVMHEALHNHYTQKSLSLSPGK

SEQ ID NO: 50 - protein, 330 aa, Artificial Sequence
  50 human XX  IgG1-E388C
ASTKGPSVFPLAPSSKSTSGGTAALGCLVKDYFPEPVTVSWNSGALTSGVHTFPAVLQSSGLYSLSSVVTVPSSSLGTQTYICNVNHKPSNTKVDKKVEPKSCDKTHTCPPCPAPELLGGPSVFLFPPKPKDTLMISRTPEVTCVVVDVSHEDPEVKFNWYVDGVEVHNAKTKPREEQYNSTYRVVSVLTVLHQDWLNGKEYKCKVSNKALPAPIEKTISKAKGQPREPQVYTLPPSREEMTKNQVSLTCLVKGFYPSDIAVEWESNGQPCNNYKTTPPVLDSDGSFFLYSKLTVDKSRWQQGNVFSCSVMHEALHNHYTQKSLSLSPGK

SEQ ID NO: 51 - protein, 330 aa, Artificial Sequence
  51 human YY  IgG1-N390C
ASTKGPSVFPLAPSSKSTSGGTAALGCLVKDYFPEPVTVSWNSGALTSGVHTFPAVLQSSGLYSLSSVVTVPSSSLGTQTYICNVNHKPSNTKVDKKVEPKSCDKTHTCPPCPAPELLGGPSVFLFPPKPKDTLMISRTPEVTCVVVDVSHEDPEVKFNWYVDGVEVHNAKTKPREEQYNSTYRVVSVLTVLHQDWLNGKEYKCKVSNKALPAPIEKTISKAKGQPREPQVYTLPPSREEMTKNQVSLTCLVKGFYPSDIAVEWESNGQPENCYKTTPPVLDSDGSFFLYSKLTVDKSRWQQGNVFSCSVMHEALHNHYTQKSLSLSPGK

SEQ ID NO: 52 - protein, 330 aa, Artificial Sequence
  52 human ZZ  IgG1-K392C
ASTKGPSVFPLAPSSKSTSGGTAALGCLVKDYFPEPVTVSWNSGALTSGVHTFPAVLQSSGLYSLSSVVTVPSSSLGTQTYICNVNHKPSNTKVDKKVEPKSCDKTHTCPPCPAPELLGGPSVFLFPPKPKDTLMISRTPEVTCVVVDVSHEDPEVKFNWYVDGVEVHNAKTKPREEQYNSTYRVVSVLTVLHQDWLNGKEYKCKVSNKALPAPIEKTISKAKGQPREPQVYTLPPSREEMTKNQVSLTCLVKGFYPSDIAVEWESNGQPENNYCTTPPVLDSDGSFFLYSKLTVDKSRWQQGNVFSCSVMHEALHNHYTQKSLSLSPGK

SEQ ID NO: 53 - protein, 330 aa, Artificial Sequences
  53 human AAA.  IgG1-T393C
ASTKGPSVFPLAPSSKSTSGGTAALGCLVKDYFPEPVTVSWNSGALTSGVHTFPAVLQSSGLYSLSSVVTVPSSSLGTQTYICNVNHKPSNTKVDKKVEPKSCDKTHTCPPCPAPELLGGPSVFLFPPKPKDTLMISRTPEVTCVVVDVSHEDPEVKFNWYVDGVEVHNAKTKPREEQYNSTYRVVSVLTVLHQDWLNGKEYKCKVSNKALPAPIEKTISKAKGQPREPQVYTLPPSREEMTKNQVSLTCLVKGFYPSDIAVEWESNGQPENNYKCTPPVLDSDGSFFLYSKLTVDKSRWQQGNVFSCSVMHEALHNHYTQKSLSLSPGK

SEQ ID NO: 54 - protein, 330 aa, Artificial Sequence
  54 human BBB  IgG1-L398C
ASTKGPSVFPLAPSSKSTSGGTAALGCLVKDYFPEPVTVSWNSGALTSGVHTFPAVLQSSGLYSLSSVVTVPSSSLGTQTYICNVNHKPSNTKVDKKVEPKSCDKTHTCPPCPAPELLGGPSVFLFPPKPKDTLMISRTPEVTCVVVDVSHEDPEVKFNWYVDGVEVHNAKTKPREEQYNSTYRVVSVLTVLHQDWLNGKEYKCKVSNKALPAPIEKTISKAKGQPREPQVYTLPPSREEMTKNQVSLTCLVKGFYPSDIAVEWESNGQPENNYKTTPPVCDSDGSFFLYSKLTVDKSRWQQGNVFSCSVMHEALHNHYTQKSLSLSPGK

SEQ ID NO: 55 - protein, 330 aa, Artificial Sequence
  55 human CCC.  IgG1-D401C
ASTKGPSVFPLAPSSKSTSGGTAALGCLVKDYFPEPVTVSWNSGALTSGVHTFPAVLQSSGLYSLSSVVTVPSSSLGTQTYICNVNHKPSNTKVDKKVEPKSCDKTHTCPPCPAPELLGGPSVFLFPPKPKDTLMISRTPEVTCVVVDVSHEDPEVKFNWYVDGVEVHNAKTKPREEQYNSTYRVVSVLTVLHQDWLNGKEYKCKVSNKALPAPIEKTISKAKGQPREPQVYTLPPSREEMTKNQVSLTCLVKGFYPSDIAVEWESNGQPENNYKTTPPVLDSCGSFFLYSKLTVDKSRWQQGNVFSCSVMHEALHNHYTQKSLSLSPGK

SEQ ID NO: 56 - protein, 330 aa, Artificial Sequence
  56 human DDD  IgG1-F404C
ASTKGPSVFPLAPSSKSTSGGTAALGCLVKDYFPEPVTVSWNSGALTSGVHTFPAVLQSSGLYSLSSVVTVPSSSLGTQTYICNVNHKPSNTKVDKKVEPKSCDKTHTCPPCPAPELLGGPSVFLFPPKPKDTLMISRTPEVTCVVVDVSHEDPEVKFNWYVDGVEVHNAKTKPREEQYNSTYRVVSVLTVLHQDWLNGKEYKCKVSNKALPAPIEKTISKAKGQPREPQVYTLPPSREEMTKNQVSLTCLVKGFYPSDIAVEWESNGQPENNYKTTPPVLDSDGSCFLYSKLTVDKSRWQQGNVFSCSVMHEALHNHYTQKSLSLSPGK

SEQ ID NO: 57 - protein, 330 aa, Artificial Sequence
  57 human EEE  IgG1-T411C
ASTKGPSVFPLAPSSKSTSGGTAALGCLVKDYFPEPVTVSWNSGALTSGVHTFPAVLQSSGLYSLSSVVTVPSSSLGTQTYICNVNHKPSNTKVDKKVEPKSCDKTHTCPPCPAPELLGGPSVFLFPPKPKDTLMISRTPEVTCVVVDVSHEDPEVKFNWYVDGVEVHNAKTKPREEQYNSTYRVVSVLTVLHQDWLNGKEYKCKVSNKALPAPIEKTISKAKGQPREPQVYTLPPSREEMTKNQVSLTCLVKGFYPSDIAVEWESNGQPENNYKTTPPVLDSDGSFFLYSKLCVDKSRWQQGNVFSCSVMHEALHNHYTQKSLSLSPGK

SEQ ID NO: 58 - protein, 330 aa, Artificial Sequence
  58 human FFF.  IgG1-D413C
ASTKGPSVFPLAPSSKSTSGGTAALGCLVKDYFPEPVTVSWNSGALTSGVHTFPAVLQSSGLYSLSSVVTVPSSSLGTQTYICNVNHKPSNTKVDKKVEPKSCDKTHTCPPCPAPELLGGPSVFLFPPKPKDTLMISRTPEVTCVVVDVSHEDPEVKFNWYVDGVEVHNAKTKPREEQYNSTYRVVSVLTVLHQDWLNGKEYKCKVSNKALPAPIEKTISKAKGQPREPQVYTLPPSREEMTKNQVSLTCLVKGFYPSDIAVEWESNGQPENNYKTTPPVLDSDGSFFLYSKLTVCKSRWQQGNVFSCSVMHEALHNHYTQKSLSLSPGK

SEQ ID NO: 59 - protein, 330 aa, Artificial Sequence
  59 human GGG  IgG1-K414C
ASTKGPSVFPLAPSSKSTSGGTAALGCLVKDYFPEPVTVSWNSGALTSGVHTFPAVLQSSGLYSLSSVVTVPSSSLGTQTYICNVNHKPSNTKVDKKVEPKSCDKTHTCPPCPAPELLGGPSVFLFPPKPKDTLMISRTPEVTCVVVDVSHEDPEVKFNWYVDGVEVHNAKTKPREEQYNSTYRVVSVLTVLHQDWLNGKEYKCKVSNKALPAPIEKTISKAKGQPREPQVYTLPPSREEMTKNQVSLTCLVKGFYPSDIAVEWESNGQPENNYKTTPPVLDSDGSFFLYSKLTVDCSRWQQGNVFSCSVMHEALHNHYTQKSLSLSPGK

SEQ ID NO: 60 - protein, 330 aa, Artificial Sequence
  60 human HHH  IgG1-R416C
ASTKGPSVFPLAPSSKSTSGGTAALGCLVKDYFPEPVTVSWNSGALTSGVHTFPAVLQSSGLYSLSSVVTVPSSSLGTQTYICNVNHKPSNTKVDKKVEPKSCDKTHTCPPCPAPELLGGPSVFLFPPKPKDTLMISRTPEVTCVVVDVSHEDPEVKFNWYVDGVEVHNAKTKPREEQYNSTYRVVSVLTVLHQDWLNGKEYKCKVSNKALPAPIEKTISKAKGQPREPQVYTLPPSREEMTKNQVSLTCLVKGFYPSDIAVEWESNGQPENNYKTTPPVLDSDGSFFLYSKLTVDKSCWQQGNVFSCSVMHEALHNHYTQKSLSLSPGK

SEQ ID NO: 61 - protein, 330 aa, Artificial Sequence
  61 human III.  IgG1-Q418C
ASTKGPSVFPLAPSSKSTSGGTAALGCLVKDYFPEPVTVSWNSGALTSGVHTFPAVLQSSGLYSLSSVVTVPSSSLGTQTYICNVNHKPSNTKVDKKVEPKSCDKTHTCPPCPAPELLGGPSVFLFPPKPKDTLMISRTPEVTCVVVDVSHEDPEVKFNWYVDGVEVHNAKTKPREEQYNSTYRVVSVLTVLHQDWLNGKEYKCKVSNKALPAPIEKTISKAKGQPREPQVYTLPPSREEMTKNQVSLTCLVKGFYPSDIAVEWESNGQPENNYKTTPPVLDSDGSFFLYSKLTVDKSRWCQGNVFSCSVMHEALHNHYTQKSLSLSPGK

SEQ ID NO: 62 - protein, 330 aa, Artificial Sequence
  62 human JJJ  IgG1-Q419
ASTKGPSVFPLAPSSKSTSGGTAALGCLVKDYFPEPVTVSWNSGALTSGVHTFPAVLQSSGLYSLSSVVTVPSSSLGTQTYICNVNHKPSNTKVDKKVEPKSCDKTHTCPPCPAPELLGGPSVFLFPPKPKDTLMISRTPEVTCVVVDVSHEDPEVKFNWYVDGVEVHNAKTKPREEQYNSTYRVVSVLTVLHQDWLNGKEYKCKVSNKALPAPIEKTISKAKGQPREPQVYTLPPSREEMTKNQVSLTCLVKGFYPSDIAVEWESNGQPENNYKTTPPVLDSDGSFFLYSKLTVDKSRWQCGNVFSCSVMHEALHNHYTQKSLSLSPGK

SEQ ID NO: 63 - protein, 330 aa, Artificial Sequence
  63 human KKK.  IgG1-N421C
ASTKGPSVFPLAPSSKSTSGGTAALGCLVKDYFPEPVTVSWNSGALTSGVHTFPAVLQSSGLYSLSSVVTVPSSSLGTQTYICNVNHKPSNTKVDKKVEPKSCDKTHTCPPCPAPELLGGPSVFLFPPKPKDTLMISRTPEVTCVVVDVSHEDPEVKFNWYVDGVEVHNAKTKPREEQYNSTYRVVSVLTVLHQDWLNGKEYKCKVSNKALPAPIEKTISKAKGQPREPQVYTLPPSREEMTKNQVSLTCLVKGFYPSDIAVEWESNGQPENNYKTTPPVLDSDGSFFLYSKLTVDKSRWQQGCVFSCSVMHEALHNHYTQKSLSLSPGK

SEQ ID NO: 64 - protein, 330 aa, Artificial Sequence
  64 human LLL  IgG1-V422C
ASTKGPSVFPLAPSSKSTSGGTAALGCLVKDYFPEPVTVSWNSGALTSGVHTFPAVLQSSGLYSLSSVVTVPSSSLGTQTYICNVNHKPSNTKVDKKVEPKSCDKTHTCPPCPAPELLGGPSVFLFPPKPKDTLMISRTPEVTCVVVDVSHEDPEVKFNWYVDGVEVHNAKTKPREEQYNSTYRVVSVLTVLHQDWLNGKEYKCKVSNKALPAPIEKTISKAKGQPREPQVYTLPPSREEMTKNQVSLTCLVKGFYPSDIAVEWESNGQPENNYKTTPPVLDSDGSFFLYSKLTVDKSRWQQGNCFSCSVMHEALHNHYTQKSLSLSPGK

SEQ ID NO: 65 - protein, 330 aa, Artificial Sequence
  65 human MMM.  IgG1-M428C
ASTKGPSVFPLAPSSKSTSGGTAALGCLVKDYFPEPVTVSWNSGALTSGVHTFPAVLQSSGLYSLSSVVTVPSSSLGTQTYICNVNHKPSNTKVDKKVEPKSCDKTHTCPPCPAPELLGGPSVFLFPPKPKDTLMISRTPEVTCVVVDVSHEDPEVKFNWYVDGVEVHNAKTKPREEQYNSTYRVVSVLTVLHQDWLNGKEYKCKVSNKALPAPIEKTISKAKGQPREPQVYTLPPSREEMTKNQVSLTCLVKGFYPSDIAVEWESNGQPENNYKTTPPVLDSDGSFFLYSKLTVDKSRWQQGNVFSCSVCHEALHNHYTQKSLSLSPGK

SEQ ID NO: 66 - protein, 330 aa, Artificial Sequence
  66 human NNN.  IgG1-A431C
ASTKGPSVFPLAPSSKSTSGGTAALGCLVKDYFPEPVTVSWNSGALTSGVHTFPAVLQSSGLYSLSSVVTVPSSSLGTQTYICNVNHKPSNTKVDKKVEPKSCDKTHTCPPCPAPELLGGPSVFLFPPKPKDTLMISRTPEVTCVVVDVSHEDPEVKFNWYVDGVEVHNAKTKPREEQYNSTYRVVSVLTVLHQDWLNGKEYKCKVSNKALPAPIEKTISKAKGQPREPQVYTLPPSREEMTKNQVSLTCLVKGFYPSDIAVEWESNGQPENNYKTTPPVLDSDGSFFLYSKLTVDKSRWQQGNVFSCSVMHECLHNHYTQKSLSLSPGK

SEQ ID NO: 67 - protein, 330 aa, Artificial Sequence
  67 human OOO.  IgG1-L432C
ASTKGPSVFPLAPSSKSTSGGTAALGCLVKDYFPEPVTVSWNSGALTSGVHTFPAVLQSSGLYSLSSVVTVPSSSLGTQTYICNVNHKPSNTKVDKKVEPKSCDKTHTCPPCPAPELLGGPSVFLFPPKPKDTLMISRTPEVTCVVVDVSHEDPEVKFNWYVDGVEVHNAKTKPREEQYNSTYRVVSVLTVLHQDWLNGKEYKCKVSNKALPAPIEKTISKAKGQPREPQVYTLPPSREEMTKNQVSLTCLVKGFYPSDIAVEWESNGQPENNYKTTPPVLDSDGSFFLYSKLTVDKSRWQQGNVFSCSVMHEACHNHYTQKSLSLSPGK

SEQ ID NO: 68 - protein, 330 aa, Artificial Sequence
  68 human PPP.  IgG1-T437C
ASTKGPSVFPLAPSSKSTSGGTAALGCLVKDYFPEPVTVSWNSGALTSGVHTFPAVLQSSGLYSLSSVVTVPSSSLGTQTYICNVNHKPSNTKVDKKVEPKSCDKTHTCPPCPAPELLGGPSVFLFPPKPKDTLMISRTPEVTCVVVDVSHEDPEVKFNWYVDGVEVHNAKTKPREEQYNSTYRVVSVLTVLHQDWLNGKEYKCKVSNKALPAPIEKTISKAKGQPREPQVYTLPPSREEMTKNQVSLTCLVKGFYPSDIAVEWESNGQPENNYKTTPPVLDSDGSFFLYSKLTVDKSRWQQGNVFSCSVMHEALHNHYCQKSLSLSPGK

SEQ ID NO: 69 - protein, 330 aa, Artificial Sequence
  69 human QQQ.  IgG1-Q438C
ASTKGPSVFPLAPSSKSTSGGTAALGCLVKDYFPEPVTVSWNSGALTSGVHTFPAVLQSSGLYSLSSVVTVPSSSLGTQTYICNVNHKPSNTKVDKKVEPKSCDKTHTCPPCPAPELLGGPSVFLFPPKPKDTLMISRTPEVTCVVVDVSHEDPEVKFNWYVDGVEVHNAKTKPREEQYNSTYRVVSVLTVLHQDWLNGKEYKCKVSNKALPAPIEKTISKAKGQPREPQVYTLPPSREEMTKNQVSLTCLVKGFYPSDIAVEWESNGQPENNYKTTPPVLDSDGSFFLYSKLTVDKSRWQQGNVFSCSVMHEALHNHYTCKSLSLSPGK

SEQ ID NO: 70 - protein, 330 aa, Artificial Sequence
  70 human RRR.  IgG1-K439C
ASTKGPSVFPLAPSSKSTSGGTAALGCLVKDYFPEPVTVSWNSGALTSGVHTFPAVLQSSGLYSLSSVVTVPSSSLGTQTYICNVNHKPSNTKVDKKVEPKSCDKTHTCPPCPAPELLGGPSVFLFPPKPKDTLMISRTPEVTCVVVDVSHEDPEVKFNWYVDGVEVHNAKTKPREEQYNSTYRVVSVLTVLHQDWLNGKEYKCKVSNKALPAPIEKTISKAKGQPREPQVYTLPPSREEMTKNQVSLTCLVKGFYPSDIAVEWESNGQPENNYKTTPPVLDSDGSFFLYSKLTVDKSRWQQGNVFSCSVMHEALHNHYTQCSLSLSPGK

SEQ ID NO: 71 - protein, 330 aa, 71 human SSS.  IgG1-S440C
ASTKGPSVFPLAPSSKSTSGGTAALGCLVKDYFPEPVTVSWNSGALTSGVHTFPAVLQSSGLYSLSSVVTVPSSSLGTQTYICNVNHKPSNTKVDKKVEPKSCDKTHTCPPCPAPELLGGPSVFLFPPKPKDTLMISRTPEVTCVVVDVSHEDPEVKFNWYVDGVEVHNAKTKPREEQYNSTYRVVSVLTVLHQDWLNGKEYKCKVSNKALPAPIEKTISKAKGQPREPQVYTLPPSREEMTKNQVSLTCLVKGFYPSDIAVEWESNGQPENNYKTTPPVLDSDGSFFLYSKLTVDKSRWQQGNVFSCSVMHEALHNHYTQKCLSLSPGK

SEQ ID NO: 72 - protein, 330 aa, Artificial Sequence
  72 human TTT.  IgG1-L443C
ASTKGPSVFPLAPSSKSTSGGTAALGCLVKDYFPEPVTVSWNSGALTSGVHTFPAVLQSSGLYSLSSVVTVPSSSLGTQTYICNVNHKPSNTKVDKKVEPKSCDKTHTCPPCPAPELLGGPSVFLFPPKPKDTLMISRTPEVTCVVVDVSHEDPEVKFNWYVDGVEVHNAKTKPREEQYNSTYRVVSVLTVLHQDWLNGKEYKCKVSNKALPAPIEKTISKAKGQPREPQVYTLPPSREEMTKNQVSLTCLVKGFYPSDIAVEWESNGQPENNYKTTPPVLDSDGSFFLYSKLTVDKSRWQQGNVFSCSVMHEALHNHYTQKSLSCSPGK

SEQ ID NO: 73 - protein, 330 aa, Artificial Sequence
  73 human UUU.  IgG1-S444C
ASTKGPSVFPLAPSSKSTSGGTAALGCLVKDYFPEPVTVSWNSGALTSGVHTFPAVLQSSGLYSLSSVVTVPSSSLGTQTYICNVNHKPSNTKVDKKVEPKSCDKTHTCPPCPAPELLGGPSVFLFPPKPKDTLMISRTPEVTCVVVDVSHEDPEVKFNWYVDGVEVHNAKTKPREEQYNSTYRVVSVLTVLHQDWLNGKEYKCKVSNKALPAPIEKTISKAKGQPREPQVYTLPPSREEMTKNQVSLTCLVKGFYPSDIAVEWESNGQPENNYKTTPPVLDSDGSFFLYSKLTVDKSRWQQGNVFSCSVMHEALHNHYTQKSLSLCPGK

SEQ ID NO: 74 - protein, 330 aa, Artificial Sequence
  74 human IgG1-E380C+L443C
ASTKGPSVFPLAPSSKSTSGGTAALGCLVKDYFPEPVTVSWNSGALTSGVHTFPAVLQSSGLYSLSSVVTVPSSSLGTQTYICNVNHKPSNTKVDKKVEPKSCDKTHTCPPCPAPELLGGPSVFLFPPKPKDTLMISRTPEVTCVVVDVSHEDPEVKFNWYVDGVEVHNAKTKPREEQYNSTYRVVSVLTVLHQDWLNGKEYKCKVSNKALPAPIEKTISKAKGQPREPQVYTLPPSREEMTKNQVSLTCLVKGFYPSDIAVCWESNGQPENNYKTTPPVLDSDGSFFLYSKLTVDKSRWQQGNVFSCSVMHEALHNHYTQKSLSCSPGK

SEQ ID NO: 75 - protein, 330 aa, Artificial Sequence
  75 human IgG1-L398C+L443C
ASTKGPSVFPLAPSSKSTSGGTAALGCLVKDYFPEPVTVSWNSGALTSGVHTFPAVLQSSGLYSLSSVVTVPSSSLGTQTYICNVNHKPSNTKVDKKVEPKSCDKTHTCPPCPAPELLGGPSVFLFPPKPKDTLMISRTPEVTCVVVDVSHEDPEVKFNWYVDGVEVHNAKTKPREEQYNSTYRVVSVLTVLHQDWLNGKEYKCKVSNKALPAPIEKTISKAKGQPREPQVYTLPPSREEMTKNQVSLTCLVKGFYPSDIAVEWESNGQPENNYKTTPPVCDSDGSFFLYSKLTVDKSRWQQGNVFSCSVMHEALHNHYTQKSLSCSPGK

SEQ ID NO: 76 - protein, 330 aa, Artificial Sequence
  76 human IgG1- V422C+L443C
ASTKGPSVFPLAPSSKSTSGGTAALGCLVKDYFPEPVTVSWNSGALTSGVHTFPAVLQSSGLYSLSSVVTVPSSSLGTQTYICNVNHKPSNTKVDKKVEPKSCDKTHTCPPCPAPELLGGPSVFLFPPKPKDTLMISRTPEVTCVVVDVSHEDPEVKFNWYVDGVEVHNAKTKPREEQYNSTYRVVSVLTVLHQDWLNGKEYKCKVSNKALPAPIEKTISKAKGQPREPQVYTLPPSREEMTKNQVSLTCLVKGFYPSDIAVEWESNGQPENNYKTTPPVLDSDGSFFLYSKLTVDKSRWQQGNCFSCSVMHEALHNHYTQKSLSCSPGK

SEQ ID NO: 77 - protein, 330 aa, Artificial Sequence
  77 human IgG1- E380C+L398C
ASTKGPSVFPLAPSSKSTSGGTAALGCLVKDYFPEPVTVSWNSGALTSGVHTFPAVLQSSGLYSLSSVVTVPSSSLGTQTYICNVNHKPSNTKVDKKVEPKSCDKTHTCPPCPAPELLGGPSVFLFPPKPKDTLMISRTPEVTCVVVDVSHEDPEVKFNWYVDGVEVHNAKTKPREEQYNSTYRVVSVLTVLHQDWLNGKEYKCKVSNKALPAPIEKTISKAKGQPREPQVYTLPPSREEMTKNQVSLTCLVKGFYPSDIAVCWESNGQPENNYKTTPPVCDSDGSFFLYSKLTVDKSRWQQGNVFSCSVMHEALHNHYTQKSLSLSPGK

SEQ ID NO: 78 - protein, 330 aa, Artificial Sequence
  78 human IgG1- L398C+V422C
ASTKGPSVFPLAPSSKSTSGGTAALGCLVKDYFPEPVTVSWNSGALTSGVHTFPAVLQSSGLYSLSSVVTVPSSSLGTQTYICNVNHKPSNTKVDKKVEPKSCDKTHTCPPCPAPELLGGPSVFLFPPKPKDTLMISRTPEVTCVVVDVSHEDPEVKFNWYVDGVEVHNAKTKPREEQYNSTYRVVSVLTVLHQDWLNGKEYKCKVSNKALPAPIEKTISKAKGQPREPQVYTLPPSREEMTKNQVSLTCLVKGFYPSDIAVEWESNGQPENNYKTTPPVCDSDGSFFLYSKLTVDKSRWQQGNCFSCSVMHEALHNHYTQKSLSLSPGK

SEQ ID NO: 79 - protein, 330 aa, Artificial Sequence
  79 human IgG1-E380C+V422C
ASTKGPSVFPLAPSSKSTSGGTAALGCLVKDYFPEPVTVSWNSGALTSGVHTFPAVLQSSGLYSLSSVVTVPSSSLGTQTYICNVNHKPSNTKVDKKVEPKSCDKTHTCPPCPAPELLGGPSVFLFPPKPKDTLMISRTPEVTCVVVDVSHEDPEVKFNWYVDGVEVHNAKTKPREEQYNSTYRVVSVLTVLHQDWLNGKEYKCKVSNKALPAPIEKTISKAKGQPREPQVYTLPPSREEMTKNQVSLTCLVKGFYPSDIAVCWESNGQPENNYKTTPPVLDSDGSFFLYSKLTVDKSRWQQGNCFSCSVMHEALHNHYTQKSLSLSPGK

SEQ ID NO: 80 - protein, 330 aa, Artificial Sequence
  human IgG1-K392C+L443C
ASTKGPSVFPLAPSSKSTSGGTAALGCLVKDYFPEPVTVSWNSGALTSGVHTFPAVLQSSGLYSLSSVVTVPSSSLGTQTYICNVNHKPSNTKVDKKVEPKSCDKTHTCPPCPAPELLGGPSVFLFPPKPKDTLMISRTPEVTCVVVDVSHEDPEVKFNWYVDGVEVHNAKTKPREEQYNSTYRVVSVLTVLHQDWLNGKEYKCKVSNKALPAPIEKTISKAKGQPREPQVYTLPPSREEMTKNQVSLTCLVKGFYPSDIAVEWESNGQPENNYCTTPPVLDSDGSFFLYSKLTVDKSRWQQGNVFSCSVMHEALHNHYTQKSLSCSPGK

SEQ ID NO: 81 - protein, 330 aa, human IgG1-F404C+L443C
ASTKGPSVFPLAPSSKSTSGGTAALGCLVKDYFPEPVTVSWNSGALTSGVHTFPAVLQSSGLYSLSSVVTVPSSSLGTQTYICNVNHKPSNTKVDKKVEPKSCDKTHTCPPCPAPELLGGPSVFLFPPKPKDTLMISRTPEVTCVVVDVSHEDPEVKFNWYVDGVEVHNAKTKPREEQYNSTYRVVSVLTVLHQDWLNGKEYKCKVSNKALPAPIEKTISKAKGQPREPQVYTLPPSREEMTKNQVSLTCLVKGFYPSDIAVEWESNGQPENNYKTTPPVLDSDGSCFLYSKLTVDKSRWQQGNVFSCSVMHEALHNHYTQKSLSCSPGK

SEQ ID NO: 82 - protein, 330 aa, Artificial Sequence
  82 human IgG1-K392C+F404C
ASTKGPSVFPLAPSSKSTSGGTAALGCLVKDYFPEPVTVSWNSGALTSGVHTFPAVLQSSGLYSLSSVVTVPSSSLGTQTYICNVNHKPSNTKVDKKVEPKSCDKTHTCPPCPAPELLGGPSVFLFPPKPKDTLMISRTPEVTCVVVDVSHEDPEVKFNWYVDGVEVHNAKTKPREEQYNSTYRVVSVLTVLHQDWLNGKEYKCKVSNKALPAPIEKTISKAKGQPREPQVYTLPPSREEMTKNQVSLTCLVKGFYPSDIAVEWESNGQPENNYCTTPPVLDSDGSCFLYSKLTVDKSRWQQGNVFSCSVMHEALHNHYTQKSLSLSPGK

SEQ ID NO: 83 - protein, 449 aa, Artificial Sequence
  83 anti-5T4 antibody heavy chain
EVQLVESGGGLVQPGGSLRLSCAASGYTFTNFGMNWVRQAPGKGLEWVAWINTNTGEPRYAEEFKGRFTISRDNAKNSLYLQMNSLRAEDTAVYYCARDWDGAYFFDYWGQGTLVTVSSASTKGPSVFPLAPSSKSTSGGTAALGCLVKDYFPEPVTVSWNSGALTSGVHTFPAVLQSSGLYSLSSVVTVPSSSLGTQTYICNVNHKPSNTKVDKKVEPKSCDKTHTCPPCPAPELLGGPSVFLFPPKPKDTLMISRTPEVTCVVVDVSHEDPEVKFNWYVDGVEVHNAKTKPREEQYNSTYRVVSVLTVLHQDWLNGKEYKCKVSNKALPAPIEKTISKAKGQPREPQVYTLPPSREEMTKNQVSLTCLVKGFYPSDIAVEWESNGQPENNYKTTPPVLDSDGSFFLYSKLTVDKSRWQQGNVFSCSVMHEALHNHYTQKSLSLSPGK

SEQ ID NO: 84 - protein, 214 aa, Artificial Sequence
  84 anti-5T4 antibody light chain
DIQMTQSPSSLSASVGDRVTITCKASQSVSNDVAWYQQKPGKAPKLLIYFATNRYTGVPSRFSGSGYGTDFTLTISSLQPEDFATYYCQQDYSSPWTFGQGTKVEIKRTVAAPSVFIFPPSDEQLKSGTASVVCLLNNFYPREAKVQWKVDNALQSGNSQESVTEQDSKDSTYSLSSTLTLSKADYEKHKVYACEVTHQGLSSPVTKSFNRGEC

SEQ ID NO: 85 - protein, 450 aa, Artificial Sequence
  85 anti-Her2 antibody heavy chain
EVQLVESGGGLVQPGGSLRLSCAASGFNIKDTYIHWVRQAPGKGLEWVARIYPTNGYTRYADSVKGRFTISADTSKNTAYLQMNSLRAEDTAVYYCSRWGGDGFYAMDYWGQGTLVTVSSASTKGPSVFPLAPSSKSTSGGTAALGCLVKDYFPEPVTVSWNSGALTSGVHTFPAVLQSSGLYSLSSVVTVPSSSLGTQTYICNVNHKPSNTKVDKKVEPKSCDKTHTCPPCPAPELLGGPSVFLFPPKPKDTLMISRTPEVTCVVVDVSHEDPEVKFNWYVDGVEVHNAKTKPREEQYNSTYRVVSVLTVLHQDWLNGKEYKCKVSNKALPAPIEKTISKAKGQPREPQVYTLPPSREEMTKNQVSLTCLVKGFYPSDIAVEWESNGQPENNYKTTPPVLDSDGSFFLYSKLTVDKSRWQQGNVFSCSVMHEALHNHYTQKSLSLSPGK

SEQ ID NO: 86 - protein, 214 aa, Artificial Sequence
  86 anti-Her2 light chain
DIQMTQSPSSLSASVGDRVTITCRASQDVNTAVAWYQQKPGKAPKLLIYSASFLYSGVPSRFSGSRSGTDFTLTISSLQPEDFATYYCQQHYTTPPTFGQGTKVEIKRTVAAPSVFIFPPSDEQLKSGTASVVCLLNNFYPREAKVQWKVDNALQSGNSQESVTEQDSKDSTYSLSSTLTLSKADYEKHKVYACEVTHQGLSSPVTKSFNRGEC

SEQ ID NO: 87 - protein, 446 aa, Artificial Sequence
  87 anti-VEGFR2 antibody heavy chain
EVQLVQSGGGLVKPGGSLRLSCAASGFTFSSYSMNWVRQAPGKGLEWVSSISSSSSYIYYADSVKGRFTISRDNAKNSLYLQMNSLRAEDTAVYYCARVTDAFDIWGQGTMVTVSSASTKGPSVFPLAPSSKSTSGGTAALGCLVKDYFPEPVTVSWNSGALTSGVHTFPAVLQSSGLYSLSSVVTVPSSSLGTQTYICNVNHKPSNTKVDKKVEPKSCDKTHTCPPCPAPELLGGPSVFLFPPKPKDTLMISRTPEVTCVVVDVSHEDPEVKFNWYVDGVEVHNAKTKPREEQYNSTYRVVSVLTVLHQDWLNGKEYKCKVSNKALPAPIEKTISKAKGQPREPQVYTLPPSREEMTKNQVSLTCLVKGFYPSDIAVEWESNGQPENNYKTTPPVLDSDGSFFLYSKLTVDKSRWQQGNVFSCSVMHEALHNHYTQKSLSLSPGK

SEQ ID NO: 88 - protein, 214 aa, Artificial Sequence
  88 anti-VEGFR2 light chan
DIQMTQSPSSVSASIGDRVTITCRASQGIDNWLGWYQQKPGKAPKLLIYDASNLDTGVPSRFSGSGSGTYFTLTISSLQAEDFAVYFCQQAKAFPPTFGGGTKVDIKRTVAAPSVFIFPPSDEQLKSGTASVVCLLNNFYPREAKVQWKVDNALQSGNSQESVTEQDSKDSTYSLSSTLTLSKADYEKHKVYACEVTHQGLSSPVTKSFNRGEC

SEQ ID NO: 89 - protein, 106 aa, Homo sapiens
TVAAPSVFIFPPSDEQLKSGTASVVCLLNNFYPREAKVQWKVDNALQSGNSQESVTEQDSKDSTYSLSSTLTLSKADYEKHKVYACEVTHQGLSSPVTKSFNRGEC

SEQ ID NO: 90 - protein, 106 aa, Artificial Sequences
  90 A111C-huKappa
TVCAPSVFIFPPSDEQLKSGTASVVCLLNNFYPREAKVQWKVDNALQSGNSQESVTEQDSKDSTYSLSSTLTLSKADYEKHKVYACEVTHQGLSSPVTKSFNRGEC

SEQ ID NO: 91 - protein, 106 aa, Artificial Sequence
  91 K149C-huKappa
TVAAPSVFIFPPSDEQLKSGTASVVCLLNNFYPREAKVQWCVDNALQSGNSQESVTEQDSKDSTYSLSSTLTLSKADYEKHKVYACEVTHQGLSSPVTKSFNRGEC

SEQ ID NO: 92 - protein, 106 aa, Artificial Sequence
  92 K183C-huKappa
TVAAPSVFIFPPSDEQLKSGTASVVCLLNNFYPREAKVQWKVDNALQSGNSQESVTEQDSKDSTYSLSSTLTLSCADYEKHKVYACEVTHQGLSSPVTKSFNRGEC

SEQ ID NO: 93 - protein, 106 aa, Artificial Sequence
  93 K188C-huKappa
TVAAPSVFIFPPSDEQLKSGTASVVCLLNNFYPREAKVQWKVDNALQSGNSQESVTEQDSKDSTYSLSSTLTLSKADYECHKVYACEVTHQGLSSPVTKSFNRGEC

SEQ ID NO: 94 - protein, 106 aa, Artificial Sequence
  94 K207C-huKappa
TVAAPSVFIFPPSDEQLKSGTASVVCLLNNFYPREAKVQWKVDNALQSGNSQESVTEQDSKDSTYSLSSTLTLSKADYEKHKVYACEVTHQGLSSPVTCSFNRGEC

SEQ ID NO: 95 - protein, 106 aa, Artificial Sequence
  95 N210C-huKappa
TVAAPSVFIFPPSDEQLKSGTASVVCLLNNFYPREAKVQWKVDNALQSGNSQESVTEQDSKDSTYSLSSTLTLSKADYEKHKVYACEVTHQGLSSPVTKSFCRGEC

SEQ ID NO: 96 - protein, 21 aa, Artificial Sequence
  96 Partial S254C
PPKPKDTLMICRTPEVTCVVV

SEQ ID NO: 97 - protein, 21 aa, Artificial Sequence [sequence omitted]

SEQ ID NO: 98 - protein, 21 aa, Artificial Sequence [sequence omitted]

SEQ ID NO: 99 - protein, 21 aa, Artificial Sequence [sequence omitted]

SEQ ID NO: 100 - protein, 21 aa, Artificial Sequence
  100 Partial S383C
YPSDIAVEWECNGQPENNYKT

SEQ ID NO: 101 - protein, 21 aa, Artificial Sequence
  101 Partial N384C
PSDIAVEWESCGQPENNYKTT

SEQ ID NO: 102 - protein, 21 aa, Artificial Sequence
  102 Partial K392C
ESNGQPENNYCTTPPVLDSDG

SEQ ID NO: 103 - protein, 21 aa, Artificial Sequence
  103 Partial L398C
ENNYKTTPPVCDSDGSFFLYS

SEQ ID NO: 104 - protein, 21 aa, Artificial Sequence [sequence omitted]

SEQ ID NO: 105 - protein, 21 aa, Artificial Sequence [sequence omitted]

SEQ ID NO: 106 - protein, 21 aa, Artificial Sequence
  106 Partial S440C
VMHEALHNHYTQKCLSLSPGK

SEQ ID NO: 107 - protein, 21 aa, Artificial Sequence
  107 Partial L443C
VMHEALHNHYTQKSLSCSPGK

SEQ ID NO: 108 - protein, 21 aa, Artificial Sequence
  108 Partial K246C
GGPSVFLFPPCPKDTLMISRT

SEQ ID NO: 109 - protein, 21 aa, Artificial Sequence
  109 Partial D249C
SVFLFPPKPKCTLMISRTPEV

SEQ ID NO: 110 - protein, 21 aa, Artificial Sequence
  110 Partial D265C
RTPEVTCVVVCVSHEDPEVKF

SEQ ID NO: 111 - protein, 21 aa, Artificial Sequence
  111 Partial S267C
PEVTCVVVDVCHEDPEVKFNW

SEQ ID NO: 112 - protein, 21 aa, Artificial Sequence
  112 Partial D270C
TCVVVDVSHECPEVKFNWYVD

SEQ ID NO: 113 - protein, 21 aa, Artificial Sequence
  113 Partial N276C
VSHEDPEVKFCWYVDGVEVHN

SEQ ID NO: 114 - protein, 21 aa, Artificial Sequence [sequence omitted]

SEQ ID NO: 115 - protein, 21 aa, Artificial Sequence [sequence omitted]

SEQ ID NO: 116 - protein, 21 aa, Artificial Sequence
  116 Partial V284C
KFNWYVDGVECHNAKTKPREE

SEQ ID NO: 117 - protein, 21 aa, Artificial Sequence
  117 Partial A287C
WYVDGVEVHNCKTKPREEQYN

SEQ ID NO: 118 - protein, 21 aa, Artificial Sequence
  118 Partial R292C
VEVHNAKTKPCEEQYNSTYRV

SEQ ID NO: 119 - protein, 21 aa, Artificial Sequence
  119 Partial E293C
EVHNAKTKPRCEQYNSTYRVV

SEQ ID NO: 120 - protein, 21 aa, Artificial Sequence
  120 Partial E294C
VHNAKTKPRECQYNSTYRVVS

SEQ ID NO: 121 - protein, 21 aa, Artificial Sequence
  121 Partial Y300C
KPREEQYNSTCRVVSVLTVLH

SEQ ID NO: 122 - protein, 21 aa, Artificial Sequence [sequence omitted]

SEQ ID NO: 123 - protein, 21 aa, Artificial Sequence [sequence omitted]

SEQ ID NO: 124 - protein, 21 aa, Artificial Sequence
  124 Partial L314C
SVLTVLHQDWCNGKEYKCKVS

SEQ ID NO: 125 - protein, 21 aa, Artificial Sequence
  125 Partial N315C
VLTVLHQDWLCGKEYKCKVSN

SEQ ID NO: 126 - protein, 21 aa, Artificial Sequence
  126 Partial E318C
VLHQDWLNGKCYKCKVSNKAL

SEQ ID NO: 127 - protein, 21 aa, Artificial Sequence
  127 Partial K320C
HQDWLNGKEYCCKVSNKALPA

SEQ ID NO: 128 - protein, 21 aa, Artificial Sequence
  128 Partial A327C
KEYKCKVSNKCLPAPIEKTIS

SEQ ID NO: 129 - protein, 21 aa, Artificial Sequence
  129 Partial I332C
KVSNKALPAPCEKTISKAKGQ

SEQ ID NO: 130 - protein, 21 aa, Artificial Sequence [sequence omitted]

SEQ ID NO: 131 - protein, 21 aa, Artificial Sequence
  131 Partial K334C
SNKALPAPIECTISKAKGQPR

SEQ ID NO: 132 - protein, 21 aa, Artificial Sequence [sequence omitted]

SEQ ID NO: 133 - protein, 21 aa, Artificial Sequence [sequence omitted]

SEQ ID NO: 134 - protein, 21 aa, Artificial Sequence [sequence omitted]

SEQ ID NO: 135 - protein, 21 aa, Artificial Sequence
  135 Partial S354C
REPQVYTLPPCREEMTKNQVS

SEQ ID NO: 136 - protein, 21 aa, Artificial Sequence [sequence omitted]

SEQ ID NO: 137 - protein, 21 aa, Artificial Sequence
  137 Partial M358C
VYTLPPSREECTKNQVSLTCL

SEQ ID NO: 138 - protein, 21 aa, Artificial Sequence [sequence omitted]

SEQ ID NO: 139 - protein, 21 aa, Artificial Sequences [sequence omitted]

SEQ ID NO: 140 - protein, 21 aa, Artificial Sequences [sequence omitted]

SEQ ID NO: 141 - protein, 21 aa, Artificial Sequence [sequence omitted]

SEQ ID NO: 142 - protein, 21 aa, Artificial Sequence [sequence omitted]

SEQ ID NO: 143 - protein, 21 aa, Artificial Sequence [sequence omitted]

SEQ ID NO: 144 - protein, 21 aa, Artificial Sequence
  144 Partial E382C
FYPSDIAVEWCSNGQPENNYK

SEQ ID NO: 145 - protein, 21 aa, Artificial Sequence
  145 Partial Q386C
DIAVEWESNGCPENNYKTTPP

SEQ ID NO: 146 - protein, 21 aa, Artificial Sequence
  146 Partial E388C
AVEWESNGQPCNNYKTTPPVL

SEQ ID NO: 147 - protein, 21 aa, Artificial Sequence [sequence omitted]

SEQ ID NO: 148 - protein, 21 aa, Artificial Sequence
  148 Partial T393C
SNGQPENNYKCTPPVLDSDGS

SEQ ID NO: 149 - protein, 21 aa, Artificial Sequence [sequence omitted]

SEQ ID NO: 150 - protein, 21 aa, Artificial Sequence [sequence omitted]

SEQ ID NO: 151 - protein, 21 aa, Artificial Sequence [sequence omitted]

SEQ ID NO: 152 - protein, 21 aa, Artificial Sequence
  152 Partial K414C
FFLYSKLTVDCSRWQQGNVFS

SEQ ID NO: 153 - protein, 21 aa, Artificial Sequence
  153 Partial R416C
LYSKLTVDKSCWQQGNVFSCS

SEQ ID NO: 154 - protein, 21 aa, Artificial Sequence
  154 Partial Q418C
SKLTVDKSRWCQGNVFSCSVM

SEQ ID NO: 155 - protein, 21 aa, Artificial Sequence
  155 Partial Q419C
KLTVDKSRWQCGNVFSCSVMH

SEQ ID NO: 156 - protein, 21 aa, Artificial Sequence [sequence omitted]

SEQ ID NO: 157 - protein, 21 aa, Artificial Sequence
  157 Partial M428C
QQGNVFSCSVCHEALHNHYTQ

SEQ ID NO: 158 - protein, 21 aa, Artificial Sequence
  158 Partial A431C
NVFSCSVMHECLHNHYTQKSL

SEQ ID NO: 159 - protein, 21 aa, Artificial Sequence
  159 Partial L432C
VFSCSVMHEACHNHYTQKSLS

SEQ ID NO: 160 - protein, 21 aa, Artificial Sequence
  160 Partial T437C
VMHEALHNHYCQKSLSLSPGK

SEQ ID NO: 161 - protein, 21 aa, Artificial Sequence
  161 Partial Q438C
VMHEALHNHYTCKSLSLSPGK

SEQ ID NO: 162 - protein, 21 aa, Artificial Sequence
  162 Partial K439C
VMHEALHNHYTQCSLSLSPGK

SEQ ID NO: 163 - protein, 21 aa, Artificial Sequence
  163 Partial S444C
VMHEALHNHYTQKSLSLCPGK

SEQ ID NO: 164 - protein, 21 aa, Artificial Sequence
  164 Partial A111C
TVCAPSVFIFPPSDEQLKSGT

SEQ ID NO: 165 - protein, 21 aa, Artificial Sequence
  165 Partial K149C
FYPREAKVQWCVDNALQSGNS

SEQ ID NO: 166 - protein, 21 aa, Artificial Sequence
  166 Partial K183C
YSLSSTLTLSCADYEKHKVYA

SEQ ID NO: 167 - protein, 21 aa, Artificial Sequence [sequence omitted]

SEQ ID NO: 168 - protein, 21 aa, Artificial Sequence
  168 Partial K207C
CEVTHQGLSSPVTCSFNRGEC

SEQ ID NO: 169 - protein, 21 aa, Artificial Sequence
  169 Partial N210C
CEVTHQGLSSPVTKSFCRGEC

SEQ ID NO: 170 - DNA, 318 bp, Homo sapiens
ggtcagcccaaggctgccccctcggtcactctgttcccgccctcctctgaggagcttcaagccaacaaggccacactggtgtgtctcataagtgacttctacccgggagccgtgacagtggcctggaaggcagatagcagccccgtcaaggcgggagtggagaccaccacaccctccaaacaaagcaacaacaagtacgcggccagcagctatctgagcctgacgcctgagcagtggaagtcccacagaagctacagctgccaggtcacgcatgaagggagcaccgtggagaagacagtggcccctacagaatgttca

SEQ ID NO: 171 - protein, 106 aa, Homo sapiens
GQPKAAPSVTLFPPSSEELQANKATLVCLISDFYPGAVTVAWKADSSPVKAGVETTTPSKQSNNKYAASSYLSLTPEQWKSHRSYSCQVTHEGSTVEKTVAPTECS

SEQ ID NO: 172 - protein, 106 aa, Artificial Sequence
  172 K110C-huLambda
GQPCAAPSVTLFPPSSEELQANKATLVCLISDFYPGAVTVAWKADSSPVKAGVETTTPSKQSNNKYAASSYLSLTPEQWKSHRSYSCQVTHEGSTVEKTVAPTECS

SEQ ID NO: 173 - protein, 106 aa, Artificial Sequence
  173 A111C-huLambda
GQPKCAPSVTLFPPSSEELQANKATLVCLISDFYPGAVTVAWKADSSPVKAGVETTTPSKQSNNKYAASSYLSLTPEQWKSHRSYSCQVTHEGSTVEKTVAPTECS

SEQ ID NO: 174 - protein, 106 aa, Artificial Sequence
  174 L125C-huLambda
GQPKAAPSVTLFPPSSEECQANKATLVCLISDFYPGAVTVAWKADSSPVKAGVETTTPSKQSNNKYAASSYLSLTPEQWKSHRSYSCQVTHEGSTVEKTVAPTECS

SEQ ID NO: 175 - protein, 106 aa, Artificial sequence
  K149C human lambda
GQPKAAPSVTLFPPSSEELQANKATLVCLISDFYPGAVTVAWCADSSPVKAGVETTTPSKQSNNKYAASSYLSLTPEQWKSHRSYSCQVTHEGSTVEKTVAPTECS

SEQ ID NO: 176 - protein, 106 aa, Artificial Sequence
  176 V155C-huLambda
GQPKAAPSVTLFPPSSEELQANKATLVCLISDFYPGAVTVAWKADSSPCKAGVETTTPSKQSNNKYAASSYLSLTPEQWKSHRSYSCQVTHEGSTVEKTVAPTECS

SEQ ID NO: 177 - protein, 106 aa, Artificial Sequence
  177 G158C-huLambda
GQPKAAPSVTLFPPSSEELQANKATLVCLISDFYPGAVTVAWKADSSPVKACVETTTPSKQSNNKYAASSYLSLTPEQWKSHRSYSCQVTHEGSTVEKTVAPTECS

SEQ ID NO: 178 - protein, 106 aa, Artificial Sequence
  178 T161C-huLambda
GQPKAAPSVTLFPPSSEELQANKATLVCLISDFYPGAVTVAWKADSSPVKAGVECTTPSKQSNNKYAASSYLSLTPEQWKSHRSYSCQVTHEGSTVEKTVAPTECS

SEQ ID NO: 179 - protein, 106 aa, Artificial Sequence
  179 Q185C-huLambda
GQPKAAPSVTLFPPSSEELQANKATLVCLISDFYPGAVTVAWKADSSPVKAGVETTTPSKQSNNKYAASSYLSLTPECWKSHRSYSCQVTHEGSTVEKTVAPTECS

SEQ ID NO: 180 - protein, 106 aa, Artificial Sequence
  180 S188C-huLambda
GQPKAAPSVTLFPPSSEELQANKATLVCLISDFYPGAVTVAWKADSSPVKAGVETTTPSKQSNNKYAASSYLSLTPEQWKCHRSYSCQVTHEGSTVEKTVAPTECS

SEQ ID NO: 181 - protein, 106 aa, Artificial Sequence
  181 H189C-huLambda
GQPKAAPSVTLFPPSSEELQANKATLVCLISDFYPGAVTVAWKADSSPVKAGVETTTPSKQSNNKYAASSYLSLTPEQWKSCRSYSCQVTHEGSTVEKTVAPTECS

SEQ ID NO: 182 - protein, 106 aa, Artificial Sequence
  182 S191C-huLambda
GQPKAAPSVTLFPPSSEELQANKATLVCLISDFYPGAVTVAWKADSSPVKAGVETTTPSKQSNNKYAASSYLSLTPEQWKSHRCYSCQVTHEGSTVEKTVAPTECS

SEQ ID NO: 183 - protein, 106 aa, Artificial Sequence
  183 T197C-huLambda
GQPKAAPSVTLFPPSSEELQANKATLVCLISDFYPGAVTVAWKADSSPVKAGVETTTPSKQSNNKYAASSYLSLTPEQWKSHRSYSCQVCHEGSTVEKTVAPTECS

SEQ ID NO: 184 - protein, 106 aa, Artificial Sequence
  184 V205C-huLambda
GQPKAAPSVTLFPPSSEELQANKATLVCLISDFYPGAVTVAWKADSSPVKAGVETTTPSKQSNNKYAASSYLSLTPEQWKSHRSYSCQVTHEGSTCEKTVAPTECS

SEQ ID NO: 185 - protein, 106 aa, Artificial Squence
  185 E206C-huLambda
GQPKAAPSVTLFPPSSEELQANKATLVCLISDFYPGAVTVAWKADSSPVKAGVETTTPSKQSNNKYAASSYLSLTPEQWKSHRSYSCQVTHEGSTVCKTVAPTECS

SEQ ID NO: 186 - protein, 106 aa, Artificial Sequence
  186 K207C-huLambda
GQPKAAPSVTLFPPSSEELQANKATLVCLISDFYPGAVTVAWKADSSPVKAGVETTTPSKQSNNKYAASSYLSLTPEQWKSHRSYSCQVTHEGSTVECTVAPTECS

SEQ ID NO: 187 - protein, 106 aa, Artificial Sequence
  187 T208C-huLambda
GQPKAAPSVTLFPPSSEELQANKATLVCLISDFYPGAVTVAWKADSSPVKAGVETTTPSKQSNNKYAASSYLSLTPEQWKSHRSYSCQVTHEGSTVEKCVAPTECS

SEQ ID NO: 188 - protein, 106 aa, Artificial Sequence
  188 A210C -huLambda
GQPKAAPSVTLFPPSSEELQANKATLVCLISDFYPGAVTVAWKADSSPVKAGVETTTPSKQSNNKYAASSYLSLTPEQWKSHRSYSCQVTHEGSTVEKTVCPTECS

SEQ ID NO: 189 - protein, 14 aa, Artificial Sequence
  189 Partial K110C
GQPCAAPSVTLFPP

SEQ ID NO: 190 - protein, 15 aa, Artificial Sequence
  190 Partial A11C
GQPKCAPSVTLFPPS

SEQ ID NO: 191 - protein, 21 aa, Artificial Sequence
  191 Partial L125C
VTLFPPSSEECQANKATLVCL

SEQ ID NO: 192 - protein, 21 aa, Artificial Sequence
  VTLFPPSSEECQANKATLVCL
FYPGAVTVAWCADSSPVKAGV

SEQ ID NO: 193 - protein, 21 aa, Artificial Sequence [sequence omitted]

SEQ ID NO: 194 - protein, 21 aa, Artificial Sequence [sequence omitted]

SEQ ID NO: 195 - protein, 21 aa, Artificial Sequence
  195 Partial T161C
DSSPVKAGVECTTPSKQSNNK

SEQ ID NO: 196 - protein, 21 aa, Artificial Sequence [sequence omitted]

SEQ ID NO: 197 - protein, 21 aa, Artificial Sequence
  197 Partial S188C
YLSLTPEQWKCHRSYSCQVTH

SEQ ID NO: 198 - protein, 21 aa, Artificial Sequence
  198 Partial H189C
LSLTPEQWKSCRSYSCQVTHE

SEQ ID NO: 199 - protein, 21 aa, Artificial Sequence
  199 Partial S191C
LTPEQWKSHRCYSCQVTHEGS

SEQ ID NO: 200 - protein, 21 aa, Artificial Sequence
  200 Partial T197C
EQWKSHRSYSCQVCHEGSTVE

SEQ ID NO: 201 - protein, 21 aa, Artificial Sequence
  EQWKSHRSYSCQVCHEGSTVE
SCQVTHEGSTCEKTVAPTECS

SEQ ID NO: 202 - protein, 20 aa, Artificial Sequence
  202 Partial E206C
CQVTHEGSTVCKTVAPTECS

SEQ ID NO: 203 - protein, 19 aa, Artificial Sequence
  203 Partial K207C
QVTHEGSTVECTVAPTECS

SEQ ID NO: 204 - protein, 18 aa, Artificial Sequence
  204 Partial T208C
VTHEGSTVEKCVAPTECS

SEQ ID NO: 205 - protein, 16 aa, Artificial Sequence
  205 Partial A210C
HEGSTVEKTVCPTECS